European Patent Application EP 4 793 292 A1, published August 19, 2026. Title: 多肽衍生物、其药物组合物及其用途. Applicant: 拜西欧斯（北京）生物技术有限公司. The sequence listing filed with the application follows.

SEQUENCE LISTING (52 sequences)

SEQ ID NO: 1 - protein, 35 aa, Mus musculus
  MOD_RES 35: note = I at position 35 is amidated
GRKKRRQRRRCDMAEHMERLKANDSLKLSQEYESI

SEQ ID NO: 2 - protein, 35 aa, Homo sapiens
  MOD_RES 35: note = I at position 35 is amidated
GRKKRRQRRRCDMAEHTERLKANDSLKLSQEYESI

SEQ ID NO: 3 - protein, 35 aa, synthetic construct; identical to SEQ ID NO: 1
  LIPID 27: note = Lys side-chain linked to 2-(2-(2-amino ethoxy) ethoxy) acetic acid-2-(2-(2-amino ethoxy) ethoxy)acetic acid-gamma Glutamic acid-Octadecanedioic acid
  SITE 6: note = D-arginine
  MOD_RES 35: note = I at position 35 is amidated
  SITE 2: note = D-arginine
  SITE 8: note = D-arginine

SEQ ID NO: 4 - protein, 35 aa, synthetic construct; identical to SEQ ID NO: 1
  MOD_RES 35: note = I at position 35 is amidated
  LIPID 21: note = Lys side-chain linked to 2-(2-(2-amino ethoxy) ethoxy) acetic acid-2-(2-(2-amino ethoxy) ethoxy)acetic acid-gamma Glutamic acid-Octadecanedioic acid
  SITE 6: note = D-arginine
  SITE 2: note = D-arginine
  SITE 8: note = D-arginine

SEQ ID NO: 5 - protein, 35 aa, synthetic construct
  MOD_RES 35: note = I at position 35 is amidated
  LIPID 23: note = Lys side-chain linked to 2-(2-(2-amino ethoxy) ethoxy) acetic acid-2-(2-(2-amino ethoxy) ethoxy)acetic acid-gamma Glutamic acid-Octadecanedioic acid
  SITE 6: note = D-arginine
  SITE 2: note = D-arginine
  SITE 8: note = D-arginine
GRKKRRQRRRCDMAEHMERLKAKDSLKLSQEYESI

SEQ ID NO: 6 - protein, 35 aa, synthetic construct; identical to SEQ ID NO: 1
  MOD_RES 35: note = I at position 35 is amidated
  SITE 6: note = D-arginine
  SITE 2: note = D-arginine
  SITE 8: note = D-arginine
  SITE 27: note = The side chain of the Lys is linked via an amide linkage to Glu in positon 31

SEQ ID NO: 7 - protein, 35 aa, synthetic construct; identical to SEQ ID NO: 1
  MOD_RES 35: note = I at position 35 is amidated
  SITE 6: note = D-arginine
  SITE 2: note = D-arginine
  SITE 8: note = D-arginine
  SITE 18: note = The side chain of the Glu is linked via an amide linkage to Lys in positon 21

SEQ ID NO: 8 - protein, 35 aa, synthetic construct; identical to SEQ ID NO: 2
  MOD_RES 35: note = I at position 35 is amidated
  LIPID 27: note = Lys side-chain linked to 2-(2-(2-amino ethoxy) ethoxy) acetic acid-2-(2-(2-amino ethoxy) ethoxy)acetic acid-gamma Glutamic acid-Octadecanedioic acid
  SITE 6: note = D-arginine
  SITE 2: note = D-arginine
  SITE 8: note = D-arginine

SEQ ID NO: 9 - protein, 34 aa, synthetic construct
  MOD_RES 34: note = I at position 34 is amidated
  LIPID 26: note = Lys side-chain linked to 2-(2-(2-amino ethoxy) ethoxy) acetic acid-2-(2-(2-amino ethoxy) ethoxy)acetic acid-gamma Glutamic acid-Octadecanedioic acid
  SITE 6: note = D-arginine
  SITE 2: note = D-arginine
  SITE 8: note = D-arginine
GRKKRRQRRRDMAEHTERLKANDSLKLSQEYESI

SEQ ID NO: 10 - protein, 35 aa, synthetic construct; identical to SEQ ID NO: 2
  MOD_RES 35: note = I at position 35 is amidated
  LIPID 21: note = Lys side-chain linked to 2-(2-(2-amino ethoxy) ethoxy) acetic acid-2-(2-(2-amino ethoxy) ethoxy)acetic acid-gamma Glutamic acid-Octadecanedioic acid
  SITE 6: note = D-arginine
  SITE 2: note = D-arginine
  SITE 8: note = D-arginine

SEQ ID NO: 11 - protein, 34 aa, synthetic construct; identical to SEQ ID NO: 9
  MOD_RES 34: note = I at position 34 is amidated
  LIPID 20: note = Lys side-chain linked to 2-(2-(2-amino ethoxy) ethoxy) acetic acid-2-(2-(2-amino ethoxy) ethoxy)acetic acid-gamma Glutamic acid-Octadecanedioic acid
  SITE 6: note = D-arginine
  SITE 2: note = D-arginine
  SITE 8: note = D-arginine

SEQ ID NO: 12 - protein, 35 aa, synthetic construct
  MOD_RES 35: note = I at position 35 is amidated
  LIPID 23: note = Lys side-chain linked to 2-(2-(2-amino ethoxy) ethoxy) acetic acid-2-(2-(2-amino ethoxy) ethoxy)acetic acid-gamma Glutamic acid-Octadecanedioic acid
  SITE 6: note = D-arginine
  SITE 2: note = D-arginine
  SITE 8: note = D-arginine
GRKKRRQRRRCDMAEHTERLKAKDSLKLSQEYESI

SEQ ID NO: 13 - protein, 34 aa, synthetic construct
  MOD_RES 34: note = I at position 34 is amidated
  LIPID 22: note = Lys side-chain linked to 2-(2-(2-amino ethoxy) ethoxy) acetic acid-2-(2-(2-amino ethoxy) ethoxy)acetic acid-gamma Glutamic acid-Octadecanedioic acid
  SITE 6: note = D-arginine
  SITE 2: note = D-arginine
  SITE 8: note = D-arginine
GRKKRRQRRRDMAEHTERLKAKDSLKLSQEYESI

SEQ ID NO: 14 - protein, 35 aa, synthetic construct; identical to SEQ ID NO: 2
  MOD_RES 35: note = I at position 35 is amidated
  SITE 6: note = D-arginine
  SITE 2: note = D-arginine
  SITE 8: note = D-arginine
  SITE 27: note = The side chain of the Lys is linked via an amide linkage to Glu in positon 31

SEQ ID NO: 15 - protein, 34 aa, synthetic construct; identical to SEQ ID NO: 9
  MOD_RES 34: note = I at position 34 is amidated
  SITE 6: note = D-arginine
  SITE 2: note = D-arginine
  SITE 8: note = D-arginine
  SITE 26: note = The side chain of the Lys is linked via an amide linkage to Glu in positon 30

SEQ ID NO: 16 - protein, 35 aa, synthetic construct; identical to SEQ ID NO: 2
  MOD_RES 35: note = I at position 35 is amidated
  SITE 6: note = D-arginine
  SITE 2: note = D-arginine
  SITE 8: note = D-arginine
  SITE 18: note = The side chain of the Glu is linked via an amide linkage to Lys in positon 21

SEQ ID NO: 17 - protein, 34 aa, synthetic construct; identical to SEQ ID NO: 9
  MOD_RES 34: note = I at position 34 is amidated
  SITE 6: note = D-arginine
  SITE 2: note = D-arginine
  SITE 8: note = D-arginine
  SITE 17: note = The side chain of the Glu is linked via an amide linkage to Lys in positon 20

SEQ ID NO: 18 - protein, 35 aa, synthetic construct; identical to SEQ ID NO: 2
  MOD_RES 35: note = I at position 35 is amidated
  SITE 6: note = D-arginine
  SITE 2: note = D-arginine
  SITE 8: note = D-arginine
  SITE 27: note = The side chain of the Lys is linked via an amide linkage to Glu in positon 33

SEQ ID NO: 19 - protein, 34 aa, synthetic construct; identical to SEQ ID NO: 9
  MOD_RES 34: note = I at position 34 is amidated
  SITE 6: note = D-arginine
  SITE 2: note = D-arginine
  SITE 8: note = D-arginine
  SITE 26: note = The side chain of the Lys is linked via an amide linkage to Glu in positon 32

SEQ ID NO: 20 - protein, 35 aa, synthetic construct; identical to SEQ ID NO: 2
  MOD_RES 35: note = I at position 35 is amidated
  SITE 6: note = D-arginine
  SITE 2: note = D-arginine
  SITE 8: note = D-arginine
  SITE 15: note = The side chain of the Glu is linked via an amide linkage to Lys in positon 21

SEQ ID NO: 21 - protein, 34 aa, synthetic construct; identical to SEQ ID NO: 9
  MOD_RES 34: note = I at position 34 is amidated
  SITE 6: note = D-arginine
  SITE 2: note = D-arginine
  SITE 8: note = D-arginine
  SITE 14: note = The side chain of the Glu is linked via an amide linkage to Lys in positon 20

SEQ ID NO: 22 - protein, 34 aa, synthetic construct
  MOD_RES 34: note = I at position 34 is amidated
  SITE 6: note = D-arginine
  SITE 2: note = D-arginine
  SITE 8: note = D-arginine
  SITE 29: note = The side chain of the Lys is linked via an amide linkage to Glu in positon 32
GRKKRRQRRRDMAEHTERLKANDSLKLSKEYESI

SEQ ID NO: 23 - protein, 35 aa, synthetic construct
  MOD_RES 35: note = I at position 35 is amidated
  SITE 6: note = D-arginine
  SITE 2: note = D-arginine
  SITE 8: note = D-arginine
  SITE 30: note = The side chain of the Lys is linked via an amide linkage to Glu in positon 33
GRKKRRQRRRCDMAEHTERLKANDSLKLSKEYESI

SEQ ID NO: 24 - protein, 34 aa, synthetic construct; identical to SEQ ID NO: 9
  MOD_RES 34: note = I at position 34 is amidated
  SITE 6: note = D-arginine
  SITE 2: note = D-arginine
  SITE 8: note = D-arginine
  SITE 26: note = The side chain of the Lys is linked via an amide linkage to Glu in positon 32
  SITE 17: note = The side chain of the Glu is linked via an amide linkage to Lys in positon 20

SEQ ID NO: 25 - protein, 35 aa, synthetic construct; identical to SEQ ID NO: 2
  MOD_RES 35: note = I at position 35 is amidated
  SITE 6: note = D-arginine
  SITE 2: note = D-arginine
  SITE 8: note = D-arginine
  SITE 18: note = The side chain of the Glu is linked via an amide linkage to Lys in positon 21
  SITE 27: note = The side chain of the Lys is linked via an amide linkage to Glu in positon 33

SEQ ID NO: 26 - protein, 35 aa, synthetic construct; identical to SEQ ID NO: 2
  MOD_RES 35: note = I at position 35 is amidated
  SITE 27: note = The side chain of the Lys is linked via an amide linkage to Glu in positon 31

SEQ ID NO: 27 - protein, 35 aa, synthetic construct; identical to SEQ ID NO: 2
  MOD_RES 35: note = I at position 35 is amidated
  LIPID 21: note = Lys side-chain linked to 2-(2-(2-amino ethoxy) ethoxy) acetic acid-2-(2-(2-amino ethoxy) ethoxy)acetic acid-gamma Glutamic acid-Octadecanedioic acid
  SITE 6: note = D-arginine
  SITE 2: note = D-arginine
  SITE 8: note = D-arginine
  SITE 27: note = The side chain of the Lys is linked via an amide linkage to Glu in positon 31

SEQ ID NO: 28 - protein, 34 aa, synthetic construct; identical to SEQ ID NO: 9
  MOD_RES 34: note = I at position 34 is amidated
  LIPID 20: note = Lys side-chain linked to 2-(2-(2-amino ethoxy) ethoxy) acetic acid-2-(2-(2-amino ethoxy) ethoxy)acetic acid-gamma Glutamic acid-Octadecanedioic acid
  SITE 6: note = D-arginine
  SITE 2: note = D-arginine
  SITE 8: note = D-arginine
  SITE 26: note = The side chain of the Lys is linked via an amide linkage to Glu in positon 30

SEQ ID NO: 29 - protein, 35 aa, synthetic construct; identical to SEQ ID NO: 2
  MOD_RES 35: note = I at position 35 is amidated
  LIPID 21: note = Lys side-chain linked to 2-(2-(2-amino ethoxy) ethoxy) acetic acid-2-(2-(2-amino ethoxy) ethoxy)acetic acid-gamma Glutamic acid-Octadecanedioic acid
  SITE 27: note = The side chain of the Lys is linked via an amide linkage to Glu in positon 31

SEQ ID NO: 30 - protein, 34 aa, synthetic construct; identical to SEQ ID NO: 9
  MOD_RES 34: note = I at position 34 is amidated
  LIPID 20: note = Lys side-chain linked to 2-(2-(2-amino ethoxy) ethoxy) acetic acid-2-(2-(2-amino ethoxy) ethoxy)acetic acid-gamma Glutamic acid-Octadecanedioic acid
  SITE 26: note = The side chain of the Lys is linked via an amide linkage to Glu in positon 30

SEQ ID NO: 31 - protein, 35 aa, synthetic construct; identical to SEQ ID NO: 2
  MOD_RES 35: note = I at position 35 is amidated
  LIPID 27: note = Lys side-chain linked to 2-(2-(2-amino ethoxy) ethoxy) acetic acid-2-(2-(2-amino ethoxy) ethoxy)acetic acid-gamma Glutamic acid-Octadecanedioic acid
  SITE 6: note = D-arginine
  SITE 2: note = D-arginine
  SITE 8: note = D-arginine
  SITE 18: note = The side chain of the Glu is linked via an amide linkage to Lys in positon 21

SEQ ID NO: 32 - protein, 34 aa, synthetic construct; identical to SEQ ID NO: 9
  MOD_RES 34: note = I at position 34 is amidated
  LIPID 26: note = Lys side-chain linked to 2-(2-(2-amino ethoxy) ethoxy) acetic acid-2-(2-(2-amino ethoxy) ethoxy)acetic acid-gamma Glutamic acid-Octadecanedioic acid
  SITE 6: note = D-arginine
  SITE 2: note = D-arginine
  SITE 8: note = D-arginine
  SITE 17: note = The side chain of the Glu is linked via an amide linkage to Lys in positon 20

SEQ ID NO: 33 - protein, 35 aa, synthetic construct; identical to SEQ ID NO: 2
  MOD_RES 35: note = I at position 35 is amidated
  LIPID 27: note = Lys side-chain linked to 2-(2-(2-amino ethoxy) ethoxy) acetic acid-2-(2-(2-amino ethoxy) ethoxy)acetic acid-gamma Glutamic acid-Octadecanedioic acid
  SITE 18: note = The side chain of the Glu is linked via an amide linkage to Lys in positon 21

SEQ ID NO: 34 - protein, 34 aa, synthetic construct; identical to SEQ ID NO: 9
  MOD_RES 34: note = I at position 34 is amidated
  LIPID 26: note = Lys side-chain linked to 2-(2-(2-amino ethoxy) ethoxy) acetic acid-2-(2-(2-amino ethoxy) ethoxy)acetic acid-gamma Glutamic acid-Octadecanedioic acid
  SITE 17: note = The side chain of the Glu is linked via an amide linkage to Lys in positon 20

SEQ ID NO: 35 - protein, 35 aa, synthetic construct; identical to SEQ ID NO: 2
  MOD_RES 35: note = I at position 35 is amidated
  LIPID 27: note = Lys side-chain linked to 2-(2-(2-amino ethoxy) ethoxy) acetic acid-2-(2-(2-amino ethoxy) ethoxy)acetic acid-gamma Glutamic acid-Octadecanedioic acid

SEQ ID NO: 36 - protein, 34 aa, synthetic construct; identical to SEQ ID NO: 9
  MOD_RES 34: note = I at position 34 is amidated
  LIPID 26: note = Lys side-chain linked to 2-(2-(2-amino ethoxy) ethoxy) acetic acid-2-(2-(2-amino ethoxy) ethoxy)acetic acid-gamma Glutamic acid-Octadecanedioic acid

SEQ ID NO: 37 - protein, 34 aa, synthetic construct
  MOD_RES 34: note = I at position 34 is amidated
  LIPID 26: note = Lys side-chain linked to 2-(2-(2-amino ethoxy) ethoxy) acetic acid-2-(2-(2-amino ethoxy) ethoxy)acetic acid-gamma Glutamic acid-Octadecanedioic acid
GRKKRRQRRRDMAEHMERLKANDSLKLSQEYESI

SEQ ID NO: 38 - protein, 35 aa, synthetic construct; identical to SEQ ID NO: 2
  MOD_RES 35: note = I at position 35 is amidated
  LIPID 21: note = Lys side-chain linked to 2-(2-(2-amino ethoxy) ethoxy) acetic acid-2-(2-(2-amino ethoxy) ethoxy)acetic acid-gamma Glutamic acid-Octadecanedioic acid

SEQ ID NO: 39 - protein, 34 aa, synthetic construct; identical to SEQ ID NO: 9
  MOD_RES 34: note = I at position 34 is amidated
  LIPID 20: note = Lys side-chain linked to 2-(2-(2-amino ethoxy) ethoxy) acetic acid-2-(2-(2-amino ethoxy) ethoxy)acetic acid-gamma Glutamic acid-Octadecanedioic acid

SEQ ID NO: 40 - protein, 35 aa, synthetic construct; identical to SEQ ID NO: 12
  MOD_RES 35: note = I at position 35 is amidated
  LIPID 23: note = Lys side-chain linked to 2-(2-(2-amino ethoxy) ethoxy) acetic acid-2-(2-(2-amino ethoxy) ethoxy)acetic acid-gamma Glutamic acid-Octadecanedioic acid

SEQ ID NO: 41 - protein, 34 aa, synthetic construct; identical to SEQ ID NO: 13
  MOD_RES 34: note = I at position 34 is amidated
  LIPID 22: note = Lys side-chain linked to 2-(2-(2-amino ethoxy) ethoxy) acetic acid-2-(2-(2-amino ethoxy) ethoxy)acetic acid-gamma Glutamic acid-Octadecanedioic acid

SEQ ID NO: 42 - protein, 35 aa, synthetic construct
  SITE 2: note = D-arginine
  SITE 6: note = D-arginine
  SITE 8: note = D-arginine
  SITE 27: note = The side chain of the Lys is linked via an amide linkage to Glu in positon 33
  MOD_RES 35: note = I at position 35 is amidated
GRKKRRQRRRCDMAEHTEALKANDSLKLSQEYESI

SEQ ID NO: 43 - protein, 34 aa, synthetic construct
  SITE 2: note = D-arginine
  SITE 6: note = D-arginine
  SITE 8: note = D-arginine
  SITE 26: note = The side chain of the Lys is linked via an amide linkage to Glu in positon 32
  MOD_RES 34: note = I at position 34 is amidated
GRKKRRQRRRDMAEHTEALKANDSLKLSQEYESI

SEQ ID NO: 44 - protein, 35 aa, synthetic construct; identical to SEQ ID NO: 42
  LIPID 21: note = Lys side-chain linked to 2-(2-(2-amino ethoxy) ethoxy) acetic acid-2-(2-(2-amino ethoxy) ethoxy)acetic acid-gamma Glutamic acid-Octadecanedioic acid
  MOD_RES 35: note = I at position 35 is amidated
  SITE 2: note = D-arginine
  SITE 6: note = D-arginine
  SITE 8: note = D-arginine

SEQ ID NO: 45 - protein, 34 aa, synthetic construct; identical to SEQ ID NO: 43
  LIPID 20: note = Lys side-chain linked to 2-(2-(2-amino ethoxy) ethoxy) acetic acid-2-(2-(2-amino ethoxy) ethoxy)acetic acid-gamma Glutamic acid-Octadecanedioic acid
  MOD_RES 34: note = I at position 34 is amidated
  SITE 2: note = D-arginine
  SITE 6: note = D-arginine
  SITE 8: note = D-arginine

SEQ ID NO: 46 - protein, 35 aa, synthetic construct
  MOD_RES 35: note = I at position 35 is amidated
  LIPID 19: note; note (original language) = Lys side-chain linked to 2-(2-(2-amino ethoxy) ethoxy) acetic acid-2-(2-(2-amino ethoxy) ethoxy)acetic acid-gamma Glutamic acid-Octadecanedioic acid
GRKKRRQRRRCDMAEHTEKLKANDSLKLSQEYESI

SEQ ID NO: 47 - protein, 35 aa, synthetic construct; identical to SEQ ID NO: 2
  MOD_RES 35: note = I at position 35 is amidated
  SITE 2: note = D-arginine
  SITE 6: note = D-arginine
  SITE 8: note = D-arginine
  LIPID 21: note = Lys side-chain linked to 2-(2-(2-amino ethoxy) ethoxy) acetic acid-2-(2-(2-amino ethoxy) ethoxy)acetic acid-gamma Glutamic acid-Palmitoyl

SEQ ID NO: 48 - protein, 34 aa, synthetic construct; identical to SEQ ID NO: 9
  MOD_RES 34: note = I at position 34 is amidated
  SITE 2: note = D-arginine
  SITE 6: note = D-arginine
  SITE 8: note = D-arginine
  LIPID 20: note = Lys side-chain linked to 2-(2-(2-amino ethoxy) ethoxy) acetic acid-2-(2-(2-amino ethoxy) ethoxy)acetic acid-gamma Glutamic acid-Palmitoyl

SEQ ID NO: 49 - protein, 34 aa, synthetic construct; identical to SEQ ID NO: 9
  MOD_RES 34: note = I at position 34 is amidated
  SITE 2: note = D-arginine
  SITE 6: note = D-arginine
  SITE 8: note = D-arginine
  LIPID 20: note = Lys side-chain linked to 2-(2-(2-amino ethoxy) ethoxy) acetic acid-gamma Glutamic acid-Octadecanedioic acid

SEQ ID NO: 50 - protein, 34 aa, synthetic construct; identical to SEQ ID NO: 9
  MOD_RES 34: note = I at position 34 is amidated
  SITE 2: note = D-arginine
  SITE 6: note = D-arginine
  SITE 8: note = D-arginine
  LIPID 20: note = Lys side-chain linked to 2-(2-(2-amino ethoxy) ethoxy) acetic acid-gamma Glutamic acid-Palmitoyl

SEQ ID NO: 51 - protein, 34 aa, synthetic construct; identical to SEQ ID NO: 9
  MOD_RES 34: note = I at position 34 is amidated
  SITE 2: note = D-arginine
  SITE 6: note = D-arginine
  SITE 8: note = D-arginine
  LIPID 20: note = Lys side-chain linked to 2-(2-(2-amino ethoxy) ethoxy) acetic acid-gamma Glutamic acid-Lauroyl

SEQ ID NO: 52 - protein, 11 aa, synthetic construct
GRKKRRQRRRC